European Patent Application EP 4 365 201 A1, published May 8, 2024. Title: ANTI-GFRAL ANTIBODY AND APPLICATION THEREOF. Applicant: SHANGHAI JMT-BIO TECHNOLOGY CO., LTD. The sequence listing filed with the application follows.

SEQUENCE LISTING (135 sequences)

SEQ ID NO: 1 - protein, 5 aa, Artificial Sequence
  Heavy Chain CDR1 (1)..(5)
GYGVN

SEQ ID NO: 2 - protein, 16 aa, Artificial Sequence
  Heavy Chain CDR2 (1)..(16)
MIWGDGTTDYNSALKS

SEQ ID NO: 3 - protein, 12 aa, Artificial Sequence
  Heavy Chain CDR3 (1)..(12)
DPKYNYGYAMDY

SEQ ID NO: 4 - protein, 120 aa, Artificial Sequence
  Heavy Chain Variable Region (1)..(120)
QVQLKESGPGLVAPSQSLSITCTVSGFSLTGYGVNWVRQSPGKGLEWLGMIWGDGTTDYNSALKSRLTIRKDNSKSQVFLRMNSLQTDDTARYYCARDPKYNYGYAMDYWGQGTSVTVSS

SEQ ID NO: 5 - protein, 15 aa, Artificial Sequence
  Light Chain CDR1 (1)..(15)
RASESVDNFGNSFMH

SEQ ID NO: 6 - protein, 7 aa, Artificial Sequence
  Light Chain CDR2 (1)..(7)
RASNLES

SEQ ID NO: 7 - protein, 9 aa, Artificial Sequence
  Light Chain CDR3 (1)..(9)
QQTNEEPYT

SEQ ID NO: 8 - protein, 111 aa, Artificial Sequence
  Light Chain Variable Region (1)..(111)
DIVLTQAPGSLAVSLGQRATISCRASESVDNFGNSFMHWYQQKPGQSPKLLIYRASNLESGIPARFSGSGSRTDFTLTINPVEADDVATYYCQQTNEEPYTFGGGTKLEIE

SEQ ID NO: 9 - protein, 5 aa, Artificial Sequence
  Heavy Chain CDR1 (1)..(5)
SYVIH

SEQ ID NO: 10 - protein, 17 aa, Artificial Sequence
  Heavy Chain CDR2 (1)..(17)
YINPYNDDINYNEKFKG

SEQ ID NO: 11 - protein, 9 aa, Artificial Sequence
  Heavy Chain CDR3 (1)..(9)
YDYDWYFDV

SEQ ID NO: 12 - protein, 118 aa, Artificial Sequence
  Heavy Chain Variable Region (1)..(118)
EVQLQQSGPELVKPGASVKMSCKASGYTFTSYVIHWVKQEPGQGLEWIGYINPYNDDINYNEKFKGKATLTSDKSSSTAYMEFSSLTSEDSAVYYCARYDYDWYFDVWGAGTAVTVSS

SEQ ID NO: 13 - protein, 16 aa, Artificial Sequence
  Light Chain CDR1 (1)..(16)
KSSQSLLDSDGKTYVN

SEQ ID NO: 14 - protein, 7 aa, Artificial Sequence
  Light Chain CDR2 (1)..(7)
LVSKLGS

SEQ ID NO: 15 - protein, 9 aa, Artificial Sequence
  Light Chain CDR3 (1)..(9)
WQGTHFPQT

SEQ ID NO: 16 - protein, 112 aa, Artificial Sequence
  Light Chain Variable Region (1)..(112)
DVVMTQTPLTLSVTIGQPASISCKSSQSLLDSDGKTYVNWLLQRPGQSPKRLIFLVSKLGSGVPDRFTGSGSGTDFTLKISRVEAEDLGVYYCWQGTHFPQTFGGGTKLEIK

SEQ ID NO: 17 - protein, 5 aa, Artificial Sequence
  Heavy Chain CDR1 (1)..(5)
GHGVN

SEQ ID NO: 18 - protein, 16 aa, Artificial Sequence
  Heavy Chain CDR2 (1)..(16)
MIWGDGYTDYNSALKS

SEQ ID NO: 19 - protein, 13 aa, Artificial Sequence
  Heavy Chain CDR3 (1)..(13)
DTYGRTYDYAMDY

SEQ ID NO: 20 - protein, 121 aa, Artificial Sequence
  Heavy Chain Variable Region (1)..(121)
QVQLKESGPGLVAPSQSLSITCTVSGFSLTGHGVNWVRQPPGKGLEWLGMIWGDGYTDYNSALKSRLSISKDNSKSQVFLKMNSLQTDDTATYYCARDTYGRTYDYAMDYWGQGTSVTVSS

SEQ ID NO: 21 - protein, 15 aa, Artificial Sequence
  Light Chain CDR1 (1)..(15)
RASESVDNYGNSFMH

SEQ ID NO: 22 - protein, 9 aa, Artificial Sequence
  Light Chain CDR3 (1)..(9)
QQSNEDPRT

SEQ ID NO: 23 - protein, 111 aa, Artificial Sequence
  Light Chain Variable Region (1)..(111)
DIVLTQSPASLAVSLGQRAAISCRASESVDNYGNSFMHWYQQKPGQPPKLLIYRASNLESGIPARFSGSGSRTDFTLTINPVEADDVATYYCQQSNEDPRTFGGGTKLEIK

SEQ ID NO: 24 - protein, 5 aa, Artificial Sequence
  Heavy Chain CDR1 (1)..(5)
NYWMN

SEQ ID NO: 25 - protein, 17 aa, Artificial Sequence
  Heavy Chain CDR2 (1)..(17)
QIYPGDDDADYNGKFQG

SEQ ID NO: 26 - protein, 8 aa, Artificial Sequence
  Heavy Chain CDR3 (1)..(8)
SGRRDFDY

SEQ ID NO: 27 - protein, 117 aa, Artificial Sequence
  Heavy Chain Variable Region (1)..(117)
QVQLQQSGSELVRPGSSVKISCRASGYTFSNYWMNWVKQRPGQGLEWIGQIYPGDDDADYNGKFQGKATLTADKSSSTAYMQLNTLTSEDSAVYFCTRSGRRDFDYWGQGTTLTVSS

SEQ ID NO: 28 - protein, 15 aa, Artificial Sequence
  Light Chain CDR1 (1)..(15)
RASESIDNYGNSFMH

SEQ ID NO: 29 - protein, 9 aa, Artificial Sequence
  Light Chain CDR3 (1)..(9)
QQNNEDPYT

SEQ ID NO: 30 - protein, 111 aa, Artificial Sequence
  Light Chain Variable Region (1)..(111)
NIVLTQSPASLAVSLGQRATISCRASESIDNYGNSFMHWYQQKPGQPPKLLIYRASNLESGVPARFSGSGSRTDFTLTIDPVEADDAATYYCQQNNEDPYTFGGGTKLEIK

SEQ ID NO: 31 - protein, 5 aa, Artificial Sequence
  Heavy Chain CDR1 (1)..(5)
SYGVH

SEQ ID NO: 32 - protein, 16 aa, Artificial Sequence
  Heavy Chain CDR2 (1)..(16)
VIWSGGRIDYNAAFIS

SEQ ID NO: 33 - protein, 15 aa, Artificial Sequence
  Heavy Chain CDR3 (1)..(15)
KGSSYYGLYYYGMDY

SEQ ID NO: 34 - protein, 123 aa, Artificial Sequence
  Heavy Chain Variable Region (1)..(123)
QVQLKQSGPGLVQPSQSLSITCTVSGFSLTSYGVHWVRQSPGKGLEWLGVIWSGGRIDYNAAFISRLSISKDNSKSQVFFKMNSLQADDTAIYYCARKGSSYYGLYYYGMDYWGQGTSVTVSS

SEQ ID NO: 35 - protein, 17 aa, Artificial Sequence
  Light Chain CDR1 (1)..(17)
KSSQSLLNSGNQKNYLT

SEQ ID NO: 36 - protein, 7 aa, Artificial Sequence
  Light Chain CDR2 (1)..(7)
WASTRES

SEQ ID NO: 37 - protein, 9 aa, Artificial Sequence
  Light Chain CDR3 (1)..(9)
QNDYGYPLT

SEQ ID NO: 38 - protein, 113 aa, Artificial Sequence
  Light Chain Variable Region (1)..(113)
DIVMTQSPSSLTVTAGEKVTMSCKSSQSLLNSGNQKNYLTWYQQKSGQTPKLLIYWASTRESGVPDRFTGSGSGTDFTLTISSVQAEDLAVYYCQNDYGYPLTFGAGTKLELK

SEQ ID NO: 39 - protein, 5 aa, Artificial Sequence
  Heavy Chain CDR1 (1)..(5)
GYSVN

SEQ ID NO: 40 - protein, 16 aa, Artificial Sequence
  Heavy Chain CDR2 (1)..(16)
MIWGDGSTDYNSALKS

SEQ ID NO: 41 - protein, 14 aa, Artificial Sequence
  Heavy Chain CDR3 (1)..(14)
DRDYRYDGGYIMDS

SEQ ID NO: 42 - protein, 122 aa, Artificial Sequence
  Heavy Chain Variable Region (1)..(122)
RVQLRESGPGLVAPSQSLSITCTVSGFSLTGYSVNWVRQPPGKGLEWLGMIWGDGSTDYNSALKSRLSISKDNSKSQVFLKMNSLQTDDTARYYCARDRDYRYDGGYIMDSWGQGTSVTVSS

SEQ ID NO: 43 - protein, 15 aa, Artificial Sequence
  Light Chain CDR1 (1)..(15)
RASESVDNFGNSFLH

SEQ ID NO: 44 - protein, 111 aa, Artificial Sequence
  Light Chain Variable Region (1)..(111)
DIVLTQSPGSLAVSLGQRATISCRASESVDNFGNSFLHWYQQKPGQPPKLLIYRASNLESGVPARFSGSGSRTDFTLTISPVEADDVATYYCQQSNEDPRTFGGGTKLEIR

SEQ ID NO: 45 - protein, 5 aa, Artificial Sequence
  Heavy Chain CDR1 (1)..(5)
RNWMH

SEQ ID NO: 46 - protein, 17 aa, Artificial Sequence
  Heavy Chain CDR2 (1)..(17)
EIDPSDSYTHYNQKFKG

SEQ ID NO: 47 - protein, 16 aa, Artificial Sequence
  Heavy Chain CDR3 (1)..(16)
VGNYDNGKDRLYAMDY

SEQ ID NO: 48 - protein, 125 aa, Artificial Sequence
  Heavy Chain Variable Region (1)..(125)
QVQLQQPGTEFVKPGASVKLSCKASGYTFTRNWMHWLKQRPGQGLEWIGEIDPSDSYTHYNQKFKGKATLTVDKSSSTAYMQLSSLTSEDSAVYYCARVGNYDNGKDRLYAMDYWGQGTSVTVSS

SEQ ID NO: 49 - protein, 15 aa, Artificial Sequence
  Light Chain CDR1 (1)..(15)
RASESVDNFGNTFLH

SEQ ID NO: 50 - protein, 9 aa, Artificial Sequence
  Light Chain CDR3 (1)..(9)
QQNNEDPWT

SEQ ID NO: 51 - protein, 111 aa, Artificial Sequence
  Light Chain Variable Region (1)..(111)
DIVLTQSPASLAVSLGQRATISCRASESVDNFGNTFLHWFRQKPGQPPKLLIYRASNLESGIPARFSGSGSRTDFTLTINPVEADDVATYYCQQNNEDPWTFGGGTKLEIK

SEQ ID NO: 52 - protein, 125 aa, Artificial Sequence
  Heavy Chain Variable Region (1)..(125)
QVQLQQPGTELVKPGASVKLSCKASGYTFTRNWMHWLKQRPGQGLEWIGEIDPSDSYTHYNQKFKGKATLTVEMSSSTAYMQLRSLTSEDSAVYYCARVGNYDNGTDRLYAMDYWGQGTSVTVSS

SEQ ID NO: 53 - protein, 16 aa, Artificial Sequence
  Heavy Chain CDR2 (1)..(16)
VIWSGGRTDYNAAFIS

SEQ ID NO: 54 - protein, 15 aa, Artificial Sequence
  Heavy Chain CDR3 (1)..(15)
KGSSYYGLYYYGMDF

SEQ ID NO: 55 - protein, 123 aa, Artificial Sequence
  Heavy Chain Variable Region (1)..(123)
QVQLKQSGPGLVQPSQSLSITCTVSGFSLTSYGVHWVRQSPGKGLEWLGVIWSGGRTDYNAAFISRLNISKDSSKSQVFFKMNSLQADDTAIYYCARKGSSYYGLYYYGMDFWGQGTSVTVSS

SEQ ID NO: 56 - protein, 15 aa, Artificial Sequence
  Light Chain CDR1 (1)..(15)
RASESVDNYGISFMN

SEQ ID NO: 57 - protein, 7 aa, Artificial Sequence
  Light Chain CDR2 (1)..(7)
VASNQGS

SEQ ID NO: 58 - protein, 9 aa, Artificial Sequence
  Heavy Chain CDR3 (1)..(9)
QHSKEVPRT

SEQ ID NO: 59 - protein, 111 aa, Artificial Sequence
DIVLTQSPASLTVSLGQRATISCRASESVDNYGISFMNWFQQKPGQPPKLLIYVASNQGSGVPARFSGSGSGTDFSLNIHPMEEDDTAMYFCQHSKEVPRTFGGGTKLEIK

SEQ ID NO: 60 - protein, 5 aa, Artificial Sequence
  Heavy Chain CDR1 (1)..(5)
SYAMS

SEQ ID NO: 61 - protein, 16 aa, Artificial Sequence
  Heavy Chain CDR2 (1)..(16)
SITTGGSTYYLDSVRG

SEQ ID NO: 62 - protein, 11 aa, Artificial Sequence
  Heavy Chain CDR3 (1)..(11)
SLIITATGFDY

SEQ ID NO: 63 - protein, 119 aa, Artificial Sequence
  Heavy Chain Variable Region (1)..(119)
EVKLVESGGGLVKPGGSLKLSCAASGFTFSSYAMSWVRQTPEKRLEWVASITTGGSTYYLDSVRGRFTISRDNARNILSLQMSSLRSEDTAIYYCARSLIITATGFDYWGQGTTLTVSS

SEQ ID NO: 64 - protein, 11 aa, Artificial Sequence
  Light Chain CDR1 (1)..(11)
RASQDVGTAVA

SEQ ID NO: 65 - protein, 7 aa, Artificial Sequence
  Light Chain CDR2 (1)..(7)
SASNRYT

SEQ ID NO: 66 - protein, 8 aa, Artificial Sequence
  Light Chain CDR3 (1)..(8)
QQYSIYYT

SEQ ID NO: 67 - protein, 106 aa, Artificial Sequence
  Light Chain Variable Region (1)..(106)
DIVMTQSQKFMSISVGDRVNITCRASQDVGTAVAWYQQKPGQSPKLLIYSASNRYTGVPNRFTGSGSGTDFTLAISNMQSEDLADYFCQQYSIYYTFGGGTKLEIK

SEQ ID NO: 68 - protein, 5 aa, Artificial Sequence
  Heavy Chain CDR1 (1)..(5)
SFVMS

SEQ ID NO: 69 - protein, 16 aa, Artificial Sequence
  Heavy Chain CDR2 (1)..(16)
SITSGGTTFYPDSVKG

SEQ ID NO: 70 - protein, 12 aa, Artificial Sequence
  Heavy Chain CDR3 (1)..(12)
GPPQFSSLSMDY

SEQ ID NO: 71 - protein, 120 aa, Artificial Sequence
  Heavy Chain Variable Region (1)..(120)
EVNLVESGGGLVKPGGPLKLSCAASGFTFSSFVMSWVRQTPEKRLEWVASITSGGTTFYPDSVKGRFTISRDNARNILYLQMSNLRSGDTAMYYCARGPPQFSSLSMDYWGQGTSVTVSS

SEQ ID NO: 72 - protein, 11 aa, Artificial Sequence
  Light Chain CDR1 (1)..(11)
KASQNVGTAVS

SEQ ID NO: 73 - protein, 8 aa, Artificial Sequence
  Light Chain CDR3 (1)..(8)
QQYSSLFT

SEQ ID NO: 74 - protein, 106 aa, Artificial Sequence
  Light Chain Variable Region (1)..(106)
DIVMTQSQKFMSTSVGDRITITCKASQNVGTAVSWFQQKPGQVPKLLIYSASNRYTGVPDRFTGSGSGTEFTLTISNIQSEDLADYFCQQYSSLFTFGSGTKLEIK

SEQ ID NO: 75 - protein, 10 aa, Artificial Sequence
  Heavy Chain CDR1 (1)..(10)
GYTFTDYGMN

SEQ ID NO: 76 - protein, 17 aa, Artificial Sequence
  Heavy Chain CDR2 (1)..(17)
WINTYTGEPTYADDFKD

SEQ ID NO: 77 - protein, 10 aa, Artificial Sequence
  Heavy Chain CDR3 (1)..(10)
RYGYDAGIDC

SEQ ID NO: 78 - protein, 119 aa, Artificial Sequence
  Heavy Chain Variable Region (1)..(119)
QIQLVQSGPELKKPGETVKISCKVSGYTFTDYGMNWVKQTPGKDLKWVGWINTYTGEPTYADDFKDRFAFSLEASASTAYLQINNLKNEDTATYFCARRYGYDAGIDCWGQGTTLTVSS

SEQ ID NO: 79 - protein, 15 aa, Artificial Sequence
  Light Chain CDR1 (1)..(15)
RASESVDSYGNNLMH

SEQ ID NO: 80 - protein, 7 aa, Artificial Sequence
  Light Chain CDR2 (1)..(7)
LASYLES

SEQ ID NO: 81 - protein, 111 aa, Artificial Sequence
  Light Chain Variable Region (1)..(111)
NIVLTQSPPSLAVSLGQRATISCRASESVDSYGNNLMHWYQQKPGQPPKLLIYLASYLESGVPARFSGSGSRTDFTLTIDPVEADDAATYYCQQNNEDPWTFGGGTKLEIK

SEQ ID NO: 82 - protein, 7 aa, Artificial Sequence
  Heavy Chain CDR1 (1)..(7)
TSDMGVG

SEQ ID NO: 83 - protein, 16 aa, Artificial Sequence
  Heavy Chain CDR2 (1)..(16)
HIWWDDDKYYNPSLKR

SEQ ID NO: 84 - protein, 12 aa, Artificial Sequence
  Heavy Chain CDR3 (1)..(12)
LYDYDDEYYFDY

SEQ ID NO: 85 - protein, 122 aa, Artificial Sequence
  Heavy Chain Variable Region (1)..(122)
QVTLKESGPGILKPSQTLSLTCSFSGFSLSTSDMGVGWIRQPSGKGLEWLAHIWWDDDKYYNPSLKRQLTISKDNSRNQVFLKISSVDTTDTATYYCARLYDYDDEYYFDYWGQGTTLTVSS

SEQ ID NO: 86 - protein, 11 aa, Artificial Sequence
  Light Chain CDR1 (1)..(11)
RASQDSNNYLN

SEQ ID NO: 87 - protein, 7 aa, Artificial Sequence
  Light Chain CDR2 (1)..(7)
YTSRLHS

SEQ ID NO: 88 - protein, 9 aa, Artificial Sequence
  Light Chain CDR3 (1)..(9)
QQGNTIPWT

SEQ ID NO: 89 - protein, 107 aa, Artificial Sequence
  Light Chain Variable Region (1)..(107)
DIQMTQTKSSLSASLGDRVTISCRASQDSNNYLNWYQQKPDGTVKLLIYYTSRLHSGVPSRFSGSGSGTDYSLTISNLEHEDIATYFCQQGNTIPWTFGGGTKLEIK

SEQ ID NO: 90 - protein, 120 aa, Artificial Sequence
  Heavy Chain Variable Region (1)..(120)
EVQLVESGGGLVKPGGSLRLSCAASGFTFSSFVMSWVRQAPGKGLEWVASITSGGTTFYPESVRGRFTISRDNAKNTLYLQMSSLRAEDTAVYYCARGPPQFSSLSMDYWGQGTTVTVSS

SEQ ID NO: 91 - protein, 16 aa, Artificial Sequence
  Heavy Chain CDR2 (1)..(16)
SITSGGTTFYPESVRG

SEQ ID NO: 92 - protein, 120 aa, Artificial Sequence
  Heavy Chain Variable Region (1)..(120)
EVQLVESGGGLVKPGGSLRLSCAASGFTFSSFVMSWVRQAPGKGLEWVASITSGGTTFYPDSVKGRFTISRDNAKNTLYLQMSSLRAEDTAVYYCARGPPQFSSLSMDYWGQGTTVTVSS

SEQ ID NO: 93 - protein, 120 aa, Artificial Sequence
  Heavy Chain Variable Region (1)..(120)
EVQLVESGGGLVKPGGSLRLSCAASGFTFSSFVMSWVRQAPGKGLEWVASITSGGTTFYPDSVKGRFTISRDNARNILYLQMSSLRAEDTAVYYCARGPPQFSSLSMDYWGQGTTVTVSS

SEQ ID NO: 94 - protein, 106 aa, Artificial Sequence
  Light Chain Variable Region (1)..(106)
DIQMTQSPSSLSASVGDRVTITCRASQNVGTAVSWYQQKPGKAPKLLIYSASNRYTGVPSRFSGSGSGTDFTLTISSLQPEDFATYYCQQYSSLFTFGGGTKLEIK

SEQ ID NO: 95 - protein, 11 aa, Artificial Sequence
  Light Chain CDR1 (1)..(11)
RASQNVGTAVS

SEQ ID NO: 96 - protein, 106 aa, Artificial Sequence
  Light Chain Variable Region (1)..(106)
DIQMTQSPSSLSASVGDRVTITCKASQNVGTAVSWFQQKPGKAPKLLIYSASNRYTGVPSRFSGSGSGTDFTLTISSLQPEDFATYYCQQYSSLFTFGGGTKLEIK

SEQ ID NO: 97 - protein, 106 aa, Artificial Sequence
  Light Chain Variable Region (1)..(106)
DIQMTQSPSSLSASVGDRITITCKASQNVGTAVSWFQQKPGKAPKLLIYSASNRYTGVPDRFSGSGSGTDFTLTISSLQPEDFATYYCQQYSSLFTFGGGTKLEIK

SEQ ID NO: 98 - protein, 119 aa, Artificial Sequence
  Heavy Chain Variable Region (1)..(119)
QVQLVQSGAEVKKPGASVKVSCKASGYTFTDYGMNWVRQAPGQGLEWMGWINTYTGEPTYADDFKDRVTMTTDTSTSTAYMELRSLRSDDTAVYYCARRYGYDAGIDAWGQGTLVTVSS

SEQ ID NO: 99 - protein, 10 aa, Artificial Sequence
  Heavy Chain CDR3 (1)..(10)
RYGYDAGIDA

SEQ ID NO: 100 - protein, 119 aa, Artificial Sequence
  Heavy Chain Variable Region (1)..(119)
QVQLVQSGAEVKKPGASVKVSCKASGYTFTDYGMNWVRQAPGQGLEWMGWINTYTGEPTYADDFKDRVTFTLDASTSTAYMELRSLRSDDTAVYYCARRYGYDAGIDAWGQGTLVTVSS

SEQ ID NO: 101 - protein, 119 aa, Artificial Sequence
  Heavy Chain Variable Region (1)..(119)
QVQLVQSGAEVKKPGASVKVSCKVSGYTFTDYGMNWVRQAPGQGLEWVGWINTYTGEPTYADDFKDRFTFTLDTSTSTAYMELRSLRSDDTAVYFCARRYGYDAGIDAWGQGTLVTVSS

SEQ ID NO: 102 - protein, 119 aa, Artificial Sequence
  Heavy Chain Variable Region (1)..(119)
QVQLVQSGAEVKKPGASVKISCKASGYTFTDYGMNWVRQAPGQGLEWMGWINTYTGEPTYADDFKDRVTFTLDTSTSTAYMELRSLRSDDTAVYYCARRYGYDAGIDAWGQGTLVTVSS

SEQ ID NO: 103 - protein, 119 aa, Artificial Sequence
  Heavy Chain Variable Region (1)..(119)
QVQLVQSGAEVKKPGASVKISCKASGYTFTDYGMNWVRQAPGQGLEWMGWINTYTGEPTYADDFKDRVTFTLDASTSTAYMELRSLRSDDTAVYYCARRYGYDAGIDAWGQGTLVTVSS

SEQ ID NO: 104 - protein, 119 aa, Artificial Sequence
  Heavy Chain Variable Region (1)..(119)
QVQLVQSGAEVKKPGASVKISCKASGYTFTDYGMNWVRQAPGQGLKWMGWINTYTGEPTYADDFKDRVTFTLDASTSTAYMELRSLRSDDTAVYYCARRYGYDAGIDAWGQGTLVTVSS

SEQ ID NO: 105 - protein, 119 aa, Artificial Sequence
  Heavy Chain Variable Region (1)..(119)
QVQLVQSGAEVKKPGASVKISCKVSGYTFTDYGMNWVRQTPGQGLKWVGWINTYTGEPTYADDFKDRFTFTLDASTSTAYMELRSLRSDDTAVYFCARRYGYDAGIDAWGQGTLVTVSS

SEQ ID NO: 106 - protein, 119 aa, Artificial Sequence
  Heavy Chain Variable Region (1)..(119)
QVQLVQSGAEVKKPGASVKISCKVSGYTFTDYGMNWVRQTPGQGLEWVGWINTYTGEPTYADDFKDRFTFTLDASTSTAYMELRSLRSDDTAVYFCARRYGYDAGIDAWGQGTLVTVSS

SEQ ID NO: 107 - protein, 119 aa, Artificial Sequence
  Heavy Chain Variable Region (1)..(119)
QVQLVQSGAEVKKPGASVKVSCKVSGYTFTDYGMNWVRQTPGQGLKWVGWINTYTGEPTYADDFKDRFTFTLDASTSTAYMELRSLRSDDTAVYFCARRYGYDAGIDAWGQGTLVTVSS

SEQ ID NO: 108 - protein, 119 aa, Artificial Sequence
  Heavy Chain Variable Region (1)..(119)
QVQLVQSGAEVKKPGASVKISCKVSGYTFTDYGMNWVRQAPGQGLKWVGWINTYTGEPTYADDFKDRFTFTLDASTSTAYMELRSLRSDDTAVYFCARRYGYDAGIDAWGQGTLVTVSS

SEQ ID NO: 109 - protein, 119 aa, Artificial Sequence
  Heavy Chain Variable Region (1)..(119)
QVQLVQSGAEVKKPGASVKISCKVSGYTFTDYGMNWVRQTPGQGLKWVGWINTYTGEPTYADDFKDRFTFTLDTSTSTAYMELRSLRSDDTAVYFCARRYGYDAGIDAWGQGTLVTVSS

SEQ ID NO: 110 - protein, 119 aa, Artificial Sequence
  Heavy Chain Variable Region (1)..(119)
QVQLVQSGAEVKKPGASVKVSCKVSGYTFTDYGMNWVRQAPGQGLKWVGWINTYTGEPTYADDFKDRFTFTLDASTSTAYMELRSLRSDDTAVYFCARRYGYDAGIDAWGQGTLVTVSS

SEQ ID NO: 111 - protein, 119 aa, Artificial Sequence
  Heavy Chain Variable Region (1)..(119)
QVQLVQSGAEVKKPGASVKVSCKVSGYTFTDYGMNWVRQAPGQGLEWVGWINTYTGEPTYADDFKDRFTFTLDASTSTAYMELRSLRSDDTAVYFCARRYGYDAGIDAWGQGTLVTVSS

SEQ ID NO: 112 - protein, 119 aa, Artificial Sequence
  Heavy Chain Variable Region (1)..(119)
QVQLVQSGAEVKKPGASVKISCKVSGYTFTDYGMNWVRQAPGQGLEWVGWINTYTGEPTYADDFKDRFTFTLDTSTSTAYMELRSLRSDDTAVYFCARRYGYDAGIDAWGQGTLVTVSS

SEQ ID NO: 113 - protein, 119 aa, Artificial Sequence
  Heavy Chain Variable Region (1)..(119)
QVQLVQSGAEVKKPGASVKISCKVSGYTFTDYGMNWVRQAPGQGLEWVGWINTYTGEPTYADDFKDRFTFTLDASTSTAYMELRSLRSDDTAVYFCARRYGYDAGIDAWGQGTLVTVSS

SEQ ID NO: 114 - protein, 119 aa, Artificial Sequence
  Heavy Chain Variable Region (1)..(119)
QIQLVQSGAEVKKPGASVKISCKVSGYTFTDYGMNWVRQTPGQGLKWVGWINTYTGEPTYADDFKDRFTFTLDASTSTAYLEIRSLRSDDTAVYFCARRYGYDAGIDAWGQGTLLTVSS

SEQ ID NO: 115 - protein, 119 aa, Artificial Sequence
  Heavy Chain Variable Region (1)..(119)
QVQLVQSGAEVKKPGASVKVSCKASGYTFTDYGMNWVRQAPGQGLEWMGWINTYTGEPTYAQKLQGRVTMTTDTSTSTAYMELRSLRSDDTAVYYCARRYGYDAGIDAWGQGTTVTVSS

SEQ ID NO: 116 - protein, 17 aa, Artificial Sequence
  Heavy Chain CDR2 (1)..(17)
WINTYTGEPTYAQKLQG

SEQ ID NO: 117 - protein, 119 aa, Artificial Sequence
  Heavy Chain Variable Region (1)..(119)
QVQLVQSGAEVKKPGASVKVSCKVSGYTFTDYGMNWVRQAPGQGLEWMGWINTYTGEPTYAQKLQGRVTFTTDTSTSTAYMELRSLRSDDTAVYYCARRYGYDAGIDAWGQGTTVTVSS

SEQ ID NO: 118 - protein, 119 aa, Artificial Sequence
  Heavy Chain Variable Region (1)..(119)
QVQLVQSGAEVKKPGASVKVSCKVSGYTFTDYGMNWVRQAPGQGLEWVGWINTYTGEPTYADDFKDRVTFTTDTSTSTAYMELRSLRSDDTAVYYCARRYGYDAGIDAWGQGTTVTVSS

SEQ ID NO: 119 - protein, 119 aa, Artificial Sequence
  Heavy Chain Variable Region (1)..(119)
QIQLVQSGAEVKKPGASVKISCKVSGYTFTDYGMNWVRQAPGQGLEWVGWINTYTGEPTYADDFKDRFTFTLDTSTSTAYLEIRSLRSDDTAVYYCARRYGYDAGIDAWGQGTTVTVSS

SEQ ID NO: 120 - protein, 119 aa, Artificial Sequence
  Heavy Chain Variable Region (1)..(119)
QVQLVQSGSELKKPGASVKVSCKVSGYTFTDYGMNWVRQAPGQGLEWVGWINTYTGEPTYADDFKDRFVFSLDTSVSTAYLQISSLKAEDTAVYYCARRYGYDAGIDAWGQGTTVTVSS

SEQ ID NO: 121 - protein, 119 aa, Artificial Sequence
  Heavy Chain Variable Region (1)..(119)
QIQLVQSGSELKKPGASVKISCKVSGYTFTDYGMNWVRQAPGQGLEWVGWINTYTGEPTYADDFKDRFVFSLDASVSTAYLQISSLKAEDTAVYYCARRYGYDAGIDAWGQGTTVTVSS

SEQ ID NO: 122 - protein, 111 aa, Artificial Sequence
  Light Chain Variable Region (1)..(111)
EIVLTQSPGTLSLSPGERATLSCRASESVDSYGNNLMHWYQQKPGQAPRLLIYLASYLESGIPDRFSGSGSGTDFTLTISRLEPEDFAVYYCQQNNESPWTFGQGTKVEIK

SEQ ID NO: 123 - protein, 9 aa, Artificial Sequence
  Light Chain CDR3 (1)..(9)
QQNNESPWT

SEQ ID NO: 124 - protein, 111 aa, Artificial Sequence
  Light Chain Variable Region (1)..(111)
EIVLTQSPGTLSLSPGERATLSCRASESVDSYGNNLMHWYQQKPGQAPRLLIYLASYLESGVPDRFSGSGSGTDFTLTISRLEPEDFATYYCQQNNESPWTFGQGTKVEIK

SEQ ID NO: 125 - protein, 111 aa, Artificial Sequence
  Light Chain Variable Region (1)..(111)
EIVLTQSPGTLSLSPGERATLSCRASESVDAYGNNLMHWYQQKPGQAPRLLIYLASYLESGVPDRFSGSGSGTDFTLTISRLEPEDFATYYCQQNNESPWTFGQGTKVEIK

SEQ ID NO: 126 - protein, 15 aa, Artificial Sequence
  Light Chain CDR1 (1)..(15)
RASESVDAYGNNLMH

SEQ ID NO: 127 - protein, 111 aa, Artificial Sequence
  Light Chain Variable Region (1)..(111)
EIVLTQSPGTLSLSPGERATLSCRASESVESYGNNLMHWYQQKPGQAPRLLIYLASYLESGVPDRFSGSGSGTDFTLTISRLEPEDFATYYCQQNNESPWTFGQGTKVEIK

SEQ ID NO: 128 - protein, 15 aa, Artificial Sequence
  Light Chain CDR1 (1)..(15)
RASESVESYGNNLMH

SEQ ID NO: 129 - protein, 111 aa, Artificial Sequence
  Light Chain Variable Region (1)..(111)
EIVLTQSPGTLSLSPGERATISCRASESVDSYGNNLMHWYQQKPGQAPRLLIYLASYLESGVPARFSGSGSRTDFTLTISRLEPEDFATYYCQQNNESPWTFGQGTKVEIK

SEQ ID NO: 130 - protein, 111 aa, Artificial Sequence
  Light Chain Variable Region (1)..(111)
EIVLTQSPGTLSLSPGERATISCRASESVDNYGNNLMHWYQQKPGQAPRLLIYLASYLESGVPARFSGSGSRTDFTLTISRLEPEDFATYYCQQNNESPWTFGQGTKVEIK

SEQ ID NO: 131 - protein, 111 aa, Artificial Sequence
EIVLTQSPGTLSLSPGERATISCRASESVDAYGNNLMHWYQQKPGQAPRLLIYLASYLESGVPARFSGSGSRTDFTLTISRLEPEDFATYYCQQNNESPWTFGQGTKVEIK

SEQ ID NO: 132 - protein, 111 aa, Artificial Sequence
  Light Chain Variable Region (1)..(111)
EIVLTQSPGTLSVSPGERATISCRASESVDSYGNNLMHWYQQKPGQAPRLLIYLASYLESGVPARFSGSGSRTDFTLTISRVEPEDFATYYCQQNNESPWTFGQGTKLEIK

SEQ ID NO: 133 - protein, 111 aa, Artificial Sequence
  Light Chain Variable Region (1)..(111)
DIQMTQSPSSLSASVGDRVTITCRASESVESYGNNLMHWYQQKPGKAPKLLIYLASYLESGVPSRFSGSGSGTDFTLTISSLQPEDFATYYCQQNNESPWTFGGGTKLEIK

SEQ ID NO: 134 - protein, 111 aa, Artificial Sequence
  Light Chain Variable Region (1)..(111)
DIQLTQSPSSLSASVGDRATITCRASESVDSYGNNLMHWYQQKPGKAPKLLIYLASYLESGVPSRFSGSGSGTDFTLTISSLQPEDFATYYCQQNNESPWTFGGGTKLEIK

SEQ ID NO: 135 - protein, 111 aa, Artificial Sequence
  Light Chain Variable Region (1)..(111)
DIVLTQSPASLAVSPGQRATITCRASESVDSYGNNLMHWYQQKPGQPPKLLIYLASYLESGVPARFSGSGSGTDFTLTINPVEANDTANYYCQQNNESPWTFGGGTKLEIK